European Patent Application EP 4 613 280 A1, published September 10, 2025. Title: PLANT MATERIAL FOR USE AS MEDICAMENT. Applicant: PLANTIBODIES. The sequence listing filed with the application follows.

SEQUENCE LISTING (10 sequences)

SEQ ID NO: 1 - protein, 440 aa, synthetic construct
  REGION 1..440: note = VH nivolumab
QVQLVESGGGVVQPGRSLRLDCKASGITFSNSGMHWVRQAPGKGLEWVAVIWYDGSKRYYADSVKGRFTISRDNSKNTLFLQMNSLRAEDTAVYYCATNDDYWGQGTLVTVSSASTKGPSVFPLAPCSRSTSESTAALGCLVKDYFPEPVTVSWNSGALTSGVHTFPAVLQSSGLYSLSSVVTVPSSSLGTKTYTCNVDHKPSNTKVDKRVESKYGPPCPPCPAPEFLGGPSVFLFPPKPKDTLMISRTPEVTCVVVDVSQEDPEVQFNWYVDGVEVHNAKTKPREEQFNSTYRVVSVLTVLHQDWLNGKEYKCKVSNKGLPSSIEKTISKAKGQPREPQVYTLPPSQEEMTKNQVSLTCLVKGFYPSDIAVEWESNGQPENNYKTTPPVLDSDGSFFLYSRLTVDKSRWQEGNVFSCSVMHEALHNHYTQKSLSLSLGK

SEQ ID NO: 2 - protein, 214 aa, synthetic construct
  REGION 1..214: note = VL Nivolumab
EIVLTQSPATLSLSPGERATLSCRASQSVSSYLAWYQQKPGQAPRLLIYDASNRATGIPARFSGSGSGTDFTLTISSLEPEDFAVYYCQQSSNWPRTFGQGTKVEIKRTVAAPSVFIFPPSDEQLKSGTASVVCLLNNFYPREAKVQWKVDNALQSGNSQESVTEQDSKDSTYSLSSTLTLSKADYEKHKVYACEVTHQGLSSPVTKSFNRGEC

SEQ ID NO: 3 - protein, 678 aa, synthetic construct
  REGION 1..678: note = synthetic construct
EIVLTQSPATLSLSPGERATLSCRASQSVSSYLAWYQQKPGQAPRLLIYDASNRATGIPARFSGSGSGTDFTLTISSLEPEDFAVYYCQQSSNWPRTFGQGTKVEIKRTVAAPSVFIFPPSDEQLKSGTASVVCLLNNFYPREAKVQWKVDNALQSGNSQESVTEQDSKDSTYSLSSTLTLSKADYEKHKVYACEVTHQGLSSPVTKSFNRGECHHHHHHQVQLVESGGGVVQPGRSLRLDCKASGITFSNSGMHWVRQAPGKGLEWVAVIWYDGSKRYYADSVKGRFTISRDNSKNTLFLQMNSLRAEDTAVYYCATNDDYWGQGTLVTVSSASTKGPSVFPLAPCSRSTSESTAALGCLVKDYFPEPVTVSWNSGALTSGVHTFPAVLQSSGLYSLSSVVTVPSSSLGTKTYTCNVDHKPSNTKVDKRVESKYGPPCPPCPAPEFLGGPSVFLFPPKPKDTLMISRTPEVTCVVVDVSQEDPEVQFNWYVDGVEVHNAKTKPREEQFNSTYRVVSVLTVLHQDWLNGKEYKCKVSNKGLPSSIEKTISKAKGQPREPQVYTLPPSQEEMTKNQVSLTCLVKGFYPSDIAVEWESNGQPENNYKTTPPVLDSDGSFFLYSRLTVDKSRWQEGNVFSCSVMHEALHNHYTQKSLSLSLGKYPYDVPDYAYPYDVPDYA

SEQ ID NO: 4 - DNA, 2040 bp, synthetic construct
  misc_feature 1..2040: note = nucleic acid construct
  source 1..2040: mol_type = other DNA
atggaaatcgttcttacacagtcacctgctactctttctctttcaccaggtgagagagctactctttcatgtagagctagccaatctgtttcttcttatttggcttggtatcagcaaaaacctggtcaagctcctagattgcttatctacgatgcaagtaaccgggctacaggaattcctgctagattttcaggatctggatccggtactgatttcactctcacaatttcctctttggaacctgaagatttcgctgtttattactgtcaacaatctagtaattggccaagaacttttggacagggaactaaggttgagattaaaaggactgttgctgctcctagtgtgtttatctttcctccatctgatgaacaattgaagtctggtacagcttcagtggtttgtcttcttaacaatttttaccctagagaggctaaagttcagtggaaagtggataacgctttgcaatctggtaactctcaagaatctgttactgagcaagattccaaagatagtacctactctcttagttcaacacttacattgtccaaggcagattatgagaaacataaagtgtatgcttgcgaggtgactcatcagggactctcttctcctgttactaagtcttttaacagaggagagtgtcatcaccatcatcatcatcaagttcagttggtggaaagcggaggaggagttgttcagcctggtaggtctctcagacttgattgcaaggcttctggtattacttttagtaactctggaatgcattgggttagacaagctcctggaaaaggtcttgaatgggttgctgttatttggtatgatggatctaagagatactacgctgattcagttaagggaagattcacaatttctagagataactctaaaaatactcttttccttcaaatgaattcattaagagcagaggatactgcagtgtattactgcgctaccaatgatgattattggggtcagggaacacttgttactgtttcttctgcttctactaaaggaccatctgtttttccactggctccttgttcgagatctacatctgaatcaactgcagctcttggatgtcttgttaaagattatttcccagagcctgttactgtttcttggaattctggtgctcttacatctggtgttcatacgttccctgctgttcttcaatcttctggattgtactcactctcatctgttgttacagttccttcatctagtcttggtactaaaacatatacatgtaatgttgatcataagcctagtaatactaaggttgataaaagagttgagtccaagtatggtccaccttgtccaccttgtcctgctccggagttccttggtggaccttctgtttttcttttccctccaaagcctaaggacactcttatgatttcgagaactcctgaggttacttgtgttgtggtggatgtgtcacaagaggatcctgaagttcagtttaactggtatgttgatggagttgaggttcataatgctaagactaagcctagagaagaacaattcaactctacttacagagttgtttcagtgttaactgttcttcatcaggattggcttaatggtaaggagtataagtgcaaggtttctaacaagggacttccatcatcaatagagaagactatttctaaggctaagggtcagccaagagaacctcaggtttacactcttccaccttctcaggaagaaatgactaagaaccaagtttcattaacatgtttagtcaaaggtttctacccttcagatattgctgttgagtgggaatctaatggacagcctgagaacaactataagactacaccacctgttttggattctgatggatcatttttcctttactctagattgacagtggataaatctaggtggcaagaaggaaatgttttttcttgtagtgtgatgcatgaggcgttgcataaccattacacacaaaaaagtttgtctctttcacttggtaagtatccatacgatgttcctgactatgcttatccttatgatgttccagattatgcttga

SEQ ID NO: 5 - DNA, 1965 bp, synthetic construct
  misc_feature 1..1965: note = nucleic acid construct
  source 1..1965: mol_type = other DNA
atggaaattgtgctgacccagagcccggcgaccctgagcctgagcccgggcgaacgcgcgaccctgagctgccgcgcgagccagagcgtgagcagctatctggcgtggtatcagcagaaaccgggccaggcgccgcgcctgctgatttatgatgcgagcaaccgcgcgaccggcattccggcgcgctttagcggcagcggcagcggcaccgattttaccctgaccattagcagcctggaaccggaagattttgcggtgtattattgccagcagagcagcaactggccgcgcacctttggccagggcaccaaagtggaaattaaacgcaccgtggcggcgccgagcgtgtttatttttccgccgagcgatgaacagctgaaaagcggcaccgcgagcgtggtgtgcctgctgaacaacttttatccgcgcgaagcgaaagtgcagtggaaagtggataacgcgctgcagagcggcaacagccaggaaagcgtgaccgaacaggatagcaaagatagcacctatagcctgagcagcaccctgaccctgagcaaagcggattatgaaaaacataaagtgtatgcgtgcgaagtgacccatcagggcctgagcagcccggtgaccaaaagctttaaccgcggcgaatgccaggtgcagctggtggaaagcggcggcggcgtggtgcagccgggccgcagcctgcgcctggattgcaaagcgagcggcattacctttagcaacagcggcatgcattgggtgcgccaggcgccgggcaaaggcctggaatgggtggcggtgatttggtatgatggcagcaaacgctattatgcggatagcgtgaaaggccgctttaccattagccgcgataacagcaaaaacaccctgtttctgcagatgaacagcctgcgcgcggaagataccgcggtgtattattgcgcgaccaacgatgattattggggccagggcaccctggtgaccgtgagcagcgcgagcaccaaaggcccgagcgtgtttccgctggcgccgtgcagccgcagcaccagcgaaagcaccgcggcgctgggctgcctggtgaaagattattttccggaaccggtgaccgtgagctggaacagcggcgcgctgaccagcggcgtgcatacctttccggcggtgctgcagagcagcggcctgtatagcctgagcagcgtggtgaccgtgccgagcagcagcctgggcaccaaaacctatacctgcaacgtggatcataaaccgagcaacaccaaagtggataaacgcgtggaaagcaaatatggcccgccgtgcccgccgtgcccggcgccggaatttctgggcggcccgagcgtgtttctgtttccgccgaaaccgaaagataccctgatgattagccgcaccccggaagtgacctgcgtggtggtggatgtgagccaggaagatccggaagtgcagtttaactggtatgtggatggcgtggaagtgcataacgcgaaaaccaaaccgcgcgaagaacagtttaacagcacctatcgcgtggtgagcgtgctgaccgtgctgcatcaggattggctgaacggcaaagaatataaatgcaaagtgagcaacaaaggcctgccgagcagcattgaaaaaaccattagcaaagcgaaaggccagccgcgcgaaccgcaggtgtataccctgccgccgagccaggaagaaatgaccaaaaaccaggtgagcctgacctgcctggtgaaaggcttttatccgagcgatattgcggtggaatgggaaagcaacggccagccggaaaacaactataaaaccaccccgccggtgctggatagcgatggcagcttttttctgtatagccgcctgaccgtggataaaagccgctggcaggaaggcaacgtgtttagctgcagcgtgatgcatgaagcgctgcataaccattatacccagaaaagcctgagcctgagcctgggcaaa

SEQ ID NO: 6 - DNA, 2794 bp, synthetic construct
  misc_feature 1..2794: note = nucleic acid construct
  source 1..2794: mol_type = other DNA
gccaacatggtggagcacgacactctcgtctactccaagaatatcaaagatacagtctcagaagaccaaagggctattgagacttttcaacaaagggtaatatcgggaaacctcctcggattccattgcccagctatctgtcacttcatcaaaaggacagtagaaaaggaaggtggcacctacaaatgccatcattgcgataaaggaaaggctatcgttcaagatgcctctgccgacagtggtcccaaagatggacccccacccacgaggagcatcgtggaaaaagaagacgttccaaccacgtcttcaaagcaagtggattgatgtgaacatggtggagcacgacactctcgtctactccaagaatatcaaagatacagtctcagaagaccaaagggctattgagacttttcaacaaagggtaatatcgggaaacctcctcggattccattgcccagctatctgtcacttcatcaaaaggacagtagaaaaggaaggtggcacctacaaatgccatcattgcgataaaggaaaggctatcgttcaagatgcctctgccgacagtggtcccaaagatggacccccacccacgaggagcatcgtggaaaaagaagacgttccaaccacgtcttcaaagcaagtggattgatgtgatatctccactgacgtaagggatgacgcacaatcccactatccttcgcaagacccttcctctatataaggaagttcatttcatttggagaggacacgctgaatggaaatcgttcttacacagtcacctgctactctttctctttcaccaggtgagagagctactctttcatgtagagctagccaatctgtttcttcttatttggcttggtatcagcaaaaacctggtcaagctcctagattgcttatctacgatgcaagtaaccgggctacaggaattcctgctagattttcaggatctggatccggtactgatttcactctcacaatttcctctttggaacctgaagatttcgctgtttattactgtcaacaatctagtaattggccaagaacttttggacagggaactaaggttgagattaaaaggactgttgctgctcctagtgtgtttatctttcctccatctgatgaacaattgaagtctggtacagcttcagtggtttgtcttcttaacaatttttaccctagagaggctaaagttcagtggaaagtggataacgctttgcaatctggtaactctcaagaatctgttactgagcaagattccaaagatagtacctactctcttagttcaacacttacattgtccaaggcagattatgagaaacataaagtgtatgcttgcgaggtgactcatcagggactctcttctcctgttactaagtcttttaacagaggagagtgtcatcaccatcatcatcatcaagttcagttggtggaaagcggaggaggagttgttcagcctggtaggtctctcagacttgattgcaaggcttctggtattacttttagtaactctggaatgcattgggttagacaagctcctggaaaaggtcttgaatgggttgctgttatttggtatgatggatctaagagatactacgctgattcagttaagggaagattcacaatttctagagataactctaaaaatactcttttccttcaaatgaattcattaagagcagaggatactgcagtgtattactgcgctaccaatgatgattattggggtcagggaacacttgttactgtttcttctgcttctactaaaggaccatctgtttttccactggctccttgttcgagatctacatctgaatcaactgcagctcttggatgtcttgttaaagattatttcccagagcctgttactgtttcttggaattctggtgctcttacatctggtgttcatacgttccctgctgttcttcaatcttctggattgtactcactctcatctgttgttacagttccttcatctagtcttggtactaaaacatatacatgtaatgttgatcataagcctagtaatactaaggttgataaaagagttgagtccaagtatggtccaccttgtccaccttgtcctgctccggagttccttggtggaccttctgtttttcttttccctccaaagcctaaggacactcttatgatttcgagaactcctgaggttacttgtgttgtggtggatgtgtcacaagaggatcctgaagttcagtttaactggtatgttgatggagttgaggttcataatgctaagactaagcctagagaagaacaattcaactctacttacagagttgtttcagtgttaactgttcttcatcaggattggcttaatggtaaggagtataagtgcaaggtttctaacaagggacttccatcatcaatagagaagactatttctaaggctaagggtcagccaagagaacctcaggtttacactcttccaccttctcaggaagaaatgactaagaaccaagtttcattaacatgtttagtcaaaggtttctacccttcagatattgctgttgagtgggaatctaatggacagcctgagaacaactataagactacaccacctgttttggattctgatggatcatttttcctttactctagattgacagtggataaatctaggtggcaagaaggaaatgttttttcttgtagtgtgatgcatgaggcgttgcataaccattacacacaaaaaagtttgtctctttcacttggtaagtatccatacgatgttcctgactatgcttatccttatgatgttccagattatgcttga

SEQ ID NO: 7 - DNA, 2794 bp, synthetic construct
  misc_feature 1..2794: note = nucleic acid construct
  source 1..2794: mol_type = other DNA
gccaacatggtggagcacgacactctcgtctactccaagaatatcaaagatacagtctcagaagaccaaagggctattgagacttttcaacaaagggtaatatcgggaaacctcctcggattccattgcccagctatctgtcacttcatcaaaaggacagtagaaaaggaaggtggcacctacaaatgccatcattgcgataaaggaaaggctatcgttcaagatgcctctgccgacagtggtcccaaagatggacccccacccacgaggagcatcgtggaaaaagaagacgttccaaccacgtcttcaaagcaagtggattgatgtgaacatggtggagcacgacactctcgtctactccaagaatatcaaagatacagtctcagaagaccaaagggctattgagacttttcaacaaagggtaatatcgggaaacctcctcggattccattgcccagctatctgtcacttcatcaaaaggacagtagaaaaggaaggtggcacctacaaatgccatcattgcgataaaggaaaggctatcgttcaagatgcctctgccgacagtggtcccaaagatggacccccacccacgaggagcatcgtggaaaaagaagacgttccaaccacgtcttcaaagcaagtggattgatgtgatatctccactgacgtaagggatgacgcacaatcccactatccttcgcaagacccttcctctatataaggaagttcatttcatttggagaggacacgctgaatggaaattgtgctgacccagagcccggcgaccctgagcctgagcccgggcgaacgcgcgaccctgagctgccgcgcgagccagagcgtgagcagctatctggcgtggtatcagcagaaaccgggccaggcgccgcgcctgctgatttatgatgcgagcaaccgcgcgaccggcattccggcgcgctttagcggcagcggcagcggcaccgattttaccctgaccattagcagcctggaaccggaagattttgcggtgtattattgccagcagagcagcaactggccgcgcacctttggccagggcaccaaagtggaaattaaacgcaccgtggcggcgccgagcgtgtttatttttccgccgagcgatgaacagctgaaaagcggcaccgcgagcgtggtgtgcctgctgaacaacttttatccgcgcgaagcgaaagtgcagtggaaagtggataacgcgctgcagagcggcaacagccaggaaagcgtgaccgaacaggatagcaaagatagcacctatagcctgagcagcaccctgaccctgagcaaagcggattatgaaaaacataaagtgtatgcgtgcgaagtgacccatcagggcctgagcagcccggtgaccaaaagctttaaccgcggcgaatgccaccaccaccaccaccaccaggtgcagctggtggaaagcggcggcggcgtggtgcagccgggccgcagcctgcgcctggattgcaaagcgagcggcattacctttagcaacagcggcatgcattgggtgcgccaggcgccgggcaaaggcctggaatgggtggcggtgatttggtatgatggcagcaaacgctattatgcggatagcgtgaaaggccgctttaccattagccgcgataacagcaaaaacaccctgtttctgcagatgaacagcctgcgcgcggaagataccgcggtgtattattgcgcgaccaacgatgattattggggccagggcaccctggtgaccgtgagcagcgcgagcaccaaaggcccgagcgtgtttccgctggcgccgtgcagccgcagcaccagcgaaagcaccgcggcgctgggctgcctggtgaaagattattttccggaaccggtgaccgtgagctggaacagcggcgcgctgaccagcggcgtgcatacctttccggcggtgctgcagagcagcggcctgtatagcctgagcagcgtggtgaccgtgccgagcagcagcctgggcaccaaaacctatacctgcaacgtggatcataaaccgagcaacaccaaagtggataaacgcgtggaaagcaaatatggcccgccgtgcccgccgtgcccggcgccggaatttctgggcggcccgagcgtgtttctgtttccgccgaaaccgaaagataccctgatgattagccgcaccccggaagtgacctgcgtggtggtggatgtgagccaggaagatccggaagtgcagtttaactggtatgtggatggcgtggaagtgcataacgcgaaaaccaaaccgcgcgaagaacagtttaacagcacctatcgcgtggtgagcgtgctgaccgtgctgcatcaggattggctgaacggcaaagaatataaatgcaaagtgagcaacaaaggcctgccgagcagcattgaaaaaaccattagcaaagcgaaaggccagccgcgcgaaccgcaggtgtataccctgccgccgagccaggaagaaatgaccaaaaaccaggtgagcctgacctgcctggtgaaaggcttttatccgagcgatattgcggtggaatgggaaagcaacggccagccggaaaacaactataaaaccaccccgccggtgctggatagcgatggcagcttttttctgtatagccgcctgaccgtggataaaagccgctggcaggaaggcaacgtgtttagctgcagcgtgatgcatgaagcgctgcataaccattatacccagaaaagcctgagcctgagcctgggcaaatacccatacgatgttccagattacgcttatccatatgatgttccagattatgcttaa

SEQ ID NO: 8 - DNA, 2339 bp, synthetic construct
  misc_feature 1..2339: note = nucleic acid construct
  source 1..2339: mol_type = other DNA
gatcatgagcggagaattaagggagtcacgttatgacccccgccgatgacgcgggacaagccgttttacgtttggaactgacagaaccgcaacgttgaaggagccactcagccgcgggtttctggagtttaatgagctaagcacatacgtcagaaaccattattgcgcgttcaaaagtcgcctaaggtcactatcagctagcaaatatttcttgtcaaaaatgctccactgacgttccataaattcccctcggtatccaattagagtctcatattcactctcaatccaaataatctgcaatggaaattgtgctgacccagagcccggcgaccctgagcctgagcccgggcgaacgcgcgaccctgagctgccgcgcgagccagagcgtgagcagctatctggcgtggtatcagcagaaaccgggccaggcgccgcgcctgctgatttatgatgcgagcaaccgcgcgaccggcattccggcgcgctttagcggcagcggcagcggcaccgattttaccctgaccattagcagcctggaaccggaagattttgcggtgtattattgccagcagagcagcaactggccgcgcacctttggccagggcaccaaagtggaaattaaacgcaccgtggcggcgccgagcgtgtttatttttccgccgagcgatgaacagctgaaaagcggcaccgcgagcgtggtgtgcctgctgaacaacttttatccgcgcgaagcgaaagtgcagtggaaagtggataacgcgctgcagagcggcaacagccaggaaagcgtgaccgaacaggatagcaaagatagcacctatagcctgagcagcaccctgaccctgagcaaagcggattatgaaaaacataaagtgtatgcgtgcgaagtgacccatcagggcctgagcagcccggtgaccaaaagctttaaccgcggcgaatgccaccaccaccaccaccaccaggtgcagctggtggaaagcggcggcggcgtggtgcagccgggccgcagcctgcgcctggattgcaaagcgagcggcattacctttagcaacagcggcatgcattgggtgcgccaggcgccgggcaaaggcctggaatgggtggcggtgatttggtatgatggcagcaaacgctattatgcggatagcgtgaaaggccgctttaccattagccgcgataacagcaaaaacaccctgtttctgcagatgaacagcctgcgcgcggaagataccgcggtgtattattgcgcgaccaacgatgattattggggccagggcaccctggtgaccgtgagcagcgcgagcaccaaaggcccgagcgtgtttccgctggcgccgtgcagccgcagcaccagcgaaagcaccgcggcgctgggctgcctggtgaaagattattttccggaaccggtgaccgtgagctggaacagcggcgcgctgaccagcggcgtgcatacctttccggcggtgctgcagagcagcggcctgtatagcctgagcagcgtggtgaccgtgccgagcagcagcctgggcaccaaaacctatacctgcaacgtggatcataaaccgagcaacaccaaagtggataaacgcgtggaaagcaaatatggcccgccgtgcccgccgtgcccggcgccggaatttctgggcggcccgagcgtgtttctgtttccgccgaaaccgaaagataccctgatgattagccgcaccccggaagtgacctgcgtggtggtggatgtgagccaggaagatccggaagtgcagtttaactggtatgtggatggcgtggaagtgcataacgcgaaaaccaaaccgcgcgaagaacagtttaacagcacctatcgcgtggtgagcgtgctgaccgtgctgcatcaggattggctgaacggcaaagaatataaatgcaaagtgagcaacaaaggcctgccgagcagcattgaaaaaaccattagcaaagcgaaaggccagccgcgcgaaccgcaggtgtataccctgccgccgagccaggaagaaatgaccaaaaaccaggtgagcctgacctgcctggtgaaaggcttttatccgagcgatattgcggtggaatgggaaagcaacggccagccggaaaacaactataaaaccaccccgccggtgctggatagcgatggcagcttttttctgtatagccgcctgaccgtggataaaagccgctggcaggaaggcaacgtgtttagctgcagcgtgatgcatgaagcgctgcataaccattatacccagaaaagcctgagcctgagcctgggcaaatacccatacgatgttccagattacgcttatccatatgatgttccagattatgcttaa

SEQ ID NO: 9 - DNA, 9572 bp, synthetic construct
  misc_feature 1..9572: note = nucleic acid construct
  source 1..9572: mol_type = other DNA
gccaacatggtggagcacgacactctcgtctactccaagaatatcaaagatacagtctcagaagaccaaagggctattgagacttttcaacaaagggtaatatcgggaaacctcctcggattccattgcccagctatctgtcacttcatcaaaaggacagtagaaaaggaaggtggcacctacaaatgccatcattgcgataaaggaaaggctatcgttcaagatgcctctgccgacagtggtcccaaagatggacccccacccacgaggagcatcgtggaaaaagaagacgttccaaccacgtcttcaaagcaagtggattgatgtgaacatggtggagcacgacactctcgtctactccaagaatatcaaagatacagtctcagaagaccaaagggctattgagacttttcaacaaagggtaatatcgggaaacctcctcggattccattgcccagctatctgtcacttcatcaaaaggacagtagaaaaggaaggtggcacctacaaatgccatcattgcgataaaggaaaggctatcgttcaagatgcctctgccgacagtggtcccaaagatggacccccacccacgaggagcatcgtggaaaaagaagacgttccaaccacgtcttcaaagcaagtggattgatgtgatatctccactgacgtaagggatgacgcacaatcccactatccttcgcaagacccttcctctatataaggaagttcatttcatttggagaggacacgctgaacccagctttcttgtacaaagtggtagctcgaatttccccgatcgttcaaacatttggcaataaagtttcttaagattgaatcctgttgccggtcttgcgatgattatcatataatttctgttgaattacgttaagcatgtaataattaacatgtaatgcatgacgttatttatgagatgggtttttatgattagagtcccgcaattatacatttaatacgcgatagaaaacaaaatatagcgcgcaaactaggataaattatcgcgcgcggtgtcatctatgttactagatcgggaaagcttttaaactatcagtgtttgacaggatatattggcgggtaaacctaagagaaaagagcgtttattagaataatcggatatttaaaagggcgtgaaaaggtttatccgttcgtccatttgtatgtgcatgccaaccacagggttcccctcgggatcaaagtactttgatccaacccctccgctgctatagtgcagtcggcttctgacgttcagtgcagccgtcttctgaaaacgacatgtcgcacaagtcctaagttacgcgacaggctgccgccctgcccttttcctggcgttttcttgtcgcgtgttttagtcgcataaagtagaatacttgcgactagaaccggagacattacgccatgaacaagagcgccgccgctggcctgctgggctatgcccgcgtcagcaccgacgaccaggacttgaccaaccaacgggccgaactgcacgcggccggctgcaccaagctgttttccgagaagatcaccggcaccaggcgcgaccgcccggagctggccaggatgcttgaccacctacgccctggcgacgttgtgacagtgaccaggctagaccgcctggcccgcagcacccgcgacctactggacattgccgagcgcatccaggaggccggcgcgggcctgcgtagcctggcagagccgtgggccgacaccaccacgccggccggccgcatggtgttgaccgtgttcgccggcattgccgagttcgagcgttccctaatcatcgaccgcacccggagcgggcgcgaggccgccaaggcccgaggcgtgaagtttggcccccgccctaccctcaccccggcacagatcgcgcacgcccgcgagctgatcgaccaggaaggccgcaccgtgaaagaggcggctgcactgcttggcgtgcatcgctcgaccctgtaccgcgcacttgagcgcagcgaggaagtgacgcccaccgaggccaggcggcgcggtgccttccgtgaggacgcattgaccgaggccgacgccctggcggccgccgagaatgaacgccaagaggaacaagcatgaaaccgcaccaggacggccaggacgaaccgtttttcattaccgaagagatcgaggcggagatgatcgcggccgggtacgtgttcgagccgcccgcgcacgtctcaaccgtgcggctgcatgaaatcctggccggtttgtctgatgccaagctggcggcctggccggccagcttggccgctgaagaaaccgagcgccgccgtctaaaaaggtgatgtgtatttgagtaaaacagcttgcgtcatgcggtcgctgcgtatatgatgcgatgagtaaataaacaaatacgcaaggggaacgcatgaaggttatcgctgtacttaaccagaaaggcgggtcaggcaagacgaccatcgcaacccatctagcccgcgccctgcaactcgccggggccgatgttctgttagtcgattccgatccccagggcagtgcccgcgattgggcggccgtgcgggaagatcaaccgctaaccgttgtcggcatcgaccgcccgacgattgaccgcgacgtgaaggccatcggccggcgcgacttcgtagtgatcgacggagcgccccaggcggcggacttggctgtgtccgcgatcaaggcagccgacttcgtgctgattccggtgcagccaagcccttacgacatatgggccaccgccgacctggtggagctggttaagcagcgcattgaggtcacggatggaaggctacaagcggcctttgtcgtgtcgcgggcgatcaaaggcacgcgcatcggcggtgaggttgccgaggcgctggccgggtacgagctgcccattcttgagtcccgtatcacgcagcgcgtgagctacccaggcactgccgccgccggcacaaccgttcttgaatcagaacccgagggcgacgctgcccgcgaggtccaggcgctggccgctgaaattaaatcaaaactcatttgagttaatgaggtaaagagaaaatgagcaaaagcacaaacacgctaagtgccggccgtccgagcgcacgcagcagcaaggctgcaacgttggccagcctggcagacacgccagccatgaagcgggtcaactttcagttgccggcggaggatcacaccaagctgaagatgtacgcggtacgccaaggcaagaccattaccgagctgctatctgaatacatcgcgcagctaccagagtaaatgagcaaatgaataaatgagtagatgaattttagcggctaaaggaggcggcatggaaaatcaagaacaaccaggcaccgacgccgtggaatgccccatgtgtggaggaacgggcggttggccaggcgtaagcggctgggttgcctgccggccctgcaatggcactggaacccccaagcccgaggaatcggcgtgagcggtcgcaaaccatccggcccggtacaaatcggcgcggcgctgggtgatgacctggtggagaagttgaaggccgcgcaggccgcccagcggcaacgcatcgaggcagaagcacgccccggtgaatcgtggcaagcggccgctgatcgaatccgcaaagaatcccggcaaccgccggcagccggtgcgccgtcgattaggaagccgcccaagggcgacgagcaaccagattttttcgttccgatgctctatgacgtgggcacccgcgatagtcgcagcatcatggacgtggccgttttccgtctgtcgaagcgtgaccgacgagctggcgaggtgatccgctacgagcttccagacgggcacgtagaggtttccgcagggccggccggcatggccagtgtgtgggattacgacctggtactgatggcggtttcccatctaaccgaatccatgaaccgataccgggaagggaagggagacaagcccggccgcgtgttccgtccacacgttgcggacgtactcaagttctgccggcgagccgatggcggaaagcagaaagacgacctggtagaaacctgcattcggttaaacaccacgcacgttgccatgcagcgtacgaagaaggccaagaacggccgcctggtgacggtatccgagggtgaagccttgattagccgctacaagatcgtaaagagcgaaaccgggcggccggagtacatcgagatcgagctagctgattggatgtaccgcgagatcacagaaggcaagaacccggacgtgctgacggttcaccccgattactttttgatcgatcccggcatcggccgttttctctaccgcctggcacgccgcgccgcaggcaaggcagaagccagatggttgttcaagacgatctacgaacgcagtggcagcgccggagagttcaagaagttctgtttcaccgtgcgcaagctgatcgggtcaaatgacctgccggagtacgatttgaaggaggaggcggggcaggctggcccgatcctagtcatgcgctaccgcaacctgatcgagggcgaagcatccgccggttcctaatgtacggagcagatgctagggcaaattgccctagcaggggaaaaaggtcgaaaaggtctctttcctgtggatagcacgtacattgggaacccaaagccgtacattgggaaccggaacccgtacattgggaacccaaagccgtacattgggaaccggtcacacatgtaagtgactgatataaaagagaaaaaaggcgatttttccgcctaaaactctttaaaacttattaaaactcttaaaacccgcctggcctgtgcataactgtctggccagcgcacagccgaagagctgcaaaaagcgcctacccttcggtcgctgcgctccctacgccccgccgcttcgcgtcggcctatcgcggccgctggccgctcaaaaatggctggcctacggccaggcaatctaccagggcgcggacaagccgcgccgtcgccactcgaccgccggcgcccacatcaaggcaccctgcctcgcgcgtttcggtgatgacggtgaaaacctctgacacatgcagctcccggagacggtcacagcttgtctgtaagcggatgccgggagcagacaagcccgtcagggcgcgtcagcgggtgttggcgggtgtcggggcgcagccatgacccagtcacgtagcgatagcggagtgtatactggcttaactatgcggcatcagagcagattgtactgagagtgcaccatatgcggtgtgaaataccgcacagatgcgtaaggagaaaataccgcatcaggcgctcttccgcttcctcgctcactgactcgctgcgctcggtcgttcggctgcggcgagcggtatcagctcactcaaaggcggtaatacggttatccacagaatcaggggataacgcaggaaagaacatgtgagcaaaaggccagcaaaaggccaggaaccgtaaaaaggccgcgttgctggcgtttttccataggctccgcccccctgacgagcatcacaaaaatcgacgctcaagtcagaggtggcgaaacccgacaggactataaagataccaggcgtttccccctggaagctccctcgtgcgctctcctgttccgaccctgccgcttaccggatacctgtccgcctttctcccttcgggaagcgtggcgctttctcatagctcacgctgtaggtatctcagttcggtgtaggtcgttcgctccaagctgggctgtgtgcacgaaccccccgttcagcccgaccgctgcgccttatccggtaactatcgtcttgagtccaacccggtaagacacgacttatcgccactggcagcagccactggtaacaggattagcagagcgaggtatgtaggcggtgctacagagttcttgaagtggtggcctaactacggctacactagaaggacagtatttggtatctgcgctctgctgaagccagttaccttcggaaaaagagttggtagctcttgatccggcaaacaaaccaccgctggtagcggtggtttttttgtttgcaagcagcagattacgcgcagaaaaaaaggatctcaagaagatcctttgatcttttctacggggtctgacgctcagtggaacgaaaactcacgttaagggattttggtcatgcattctaggtactaaaacaattcatccagtaaaatataatattttattttctcccaatcaggcttgatccccagtaagtcaaaaaatagctcgacatactgttcttccccgatatcctccctgatcgaccggacgcagaaggcaatgtcataccacttgtccgccctgccgcttctcccaagatcaataaagccacttactttgccatctttcacaaagatgttgctgtctcccaggtcgccgtgggaaaagacaagttcctcttcgggcttttccgtctttaaaaaatcatacagctcgcgcggatctttaaatggagtgtcttcttcccagttttcgcaatccacatcggccagatcgttattcagtaagtaatccaattcggctaagcggctgtctaagctattcgtatagggacaatccgatatgtcgatggagtgaaagagcctgatgcactccgcatacagctcgataatcttttcagggctttgttcatcttcatactcttccgagcaaaggacgccatcggcctcactcatgagcagattgctccagccatcatgccgttcaaagtgcaggacctttggaacaggcagctttccttccagccatagcatcatgtccttttcccgttccacatcataggtggtccctttataccggctgtccgtcatttttaaatataggttttcattttctcccaccagcttatataccttagcaggagacattccttccgtatcttttacgcagcggtatttttcgatcagttttttcaattccggtgatattctcattttagccatttattatttccttcctcttttctacagtatttaaagataccccaagaagctaattataacaagacgaactccaattcactgttccttgcattctaaaaccttaaataccagaaaacagctttttcaaagttgttttcaaagttggcgtataacatagtatcgacggagccgattttgaaaccgcggtgatcacaggcagcaacgctctgtcatcgttacaatcaacatgctaccctccgcgagatcatccgtgtttcaaacccggcagcttagttgccgttcttccgaatagcatcggtaacatgagcaaagtctgccgccttacaacggctctcccgctgacgccgtcccggactgatgggctgcctgtatcgagtggtgattttgtgccgagctgccggtcggggagctgttggctggctggtggcaggatatattgtggtgtaaacaaattgacgcttagacaacttaataacacattgcggacgtttttaatgtactgaattaacgccgaattgaattcgagctcggtaccgggggatctggattttagtactggattttggttttaggaattagaaattttattgatagaagtattttacaaatacaaatacatactaagggtttcttatatgctcaacacatgagcgaaaccctataggaaccctaattcccttatctgggaactactcacacattattatggagaaactcgagcttgtcgatcgacagatcccggtcggcatctactctatttctttgccctcggacgagtgctggggcgtcggtttccactatcggcgagtacttctacacagccatcggtccagacggccgcgcttctgcgggcgatttgtgtacgcccgacagtcccggctccggatcggacgattgcgtcgcatcgaccctgcgcccaagctgcatcatcgaaattgccgtcaaccaagctctgatagagttggtcaagaccaatgcggagcatatacgcccggagtcgtggcgatcctgcaagctccggatgcctccgctcgaagtagcgcgtctgctgctccatacaagccaaccacggcctccagaagaagatgttggcgacctcgtattgggaatccccgaacatcgcctcgctccagtcaatgaccgctgttatgcggccattgtccgtcaggacattgttggagccgaaatccgcgtgcacgaggtgccggacttcggggcagtcctcggcccaaagcatcagctcatcgagagcctgcgcgacggacgcactgacggtgtcgtccatcacagtttgccagtgatacacatggggatcagcaatcgcgcatatgaaatcacgccatgtagtgtattgaccgattccttgcggtccgaatgggccgaacccgctcgtctggctaagatcggccgcagcgatcgcatccatagcctccgcgaccggttgtagaacagcgggcagttcggtttcaggcaggtcttgcaacgtgacaccctgtgaacggcgggagatgcaataggtcaggctctcgctaaactccccaatgtcaagcacttccggaatcgggagcgcggccgatgcaaagtgccgataaacataacgatctttgtagaaaccatcggcgcagctatttacccgcaggacatatccacgccctcctacatcgaagctgaaagcacgagattcttcgccctccgagagctgcatcaggtcggagacgctgtcgaacttttcgatcagaaacttctcgacagacgtcgcggtgagttcaggctttttcatatctcattgccccccggatctgcgaaagctcgagagagatagatttgtagagagagactggtgatttcagcgtgtcctctccaaatgaaatgaacttccttatatagaggaagggtcttgcgaaggatagtgggattgtgcgtcatcccttacgtcagtggagatatcacatcaatccacttgctttgaagacgtggttggaacgtcttctttttccacgatgctcctcgtgggtgggggtccatctttgggaccactgtcggcagaggcatcttgaacgatagcctttcctttatcgcaatgatggcatttgtaggtgccaccttccttttctactgtccttttgatgaagtgacagatagctgggcaatggaatccgaggaggtttcccgatattaccctttgttgaaaagtctcaatagccctttggtcttctgagactgtatctttgatattcttggagtagacgagagtgtcgtgctccaccatgttcacatcaatccacttgctttgaagacgtggttggaacgtcttctttttccacgatgctcctcgtgggtgggggtccatctttgggaccactgtcggcagaggcatcttgaacgatagcctttcctttatcgcaatgatggcatttgtaggtgccaccttccttttctactgtccttttgatgaagtgacagatagctgggcaatggaatccgaggaggtttcccgatattaccctttgttgaaaagtctcaatagccctttggtcttctgagactgtatctttgatattcttggagtagacgagagtgtcgtgctccaccatgttggcgtacccggggatcctctagagtcgacctgcaggcatgcaagct

SEQ ID NO: 10 - DNA, 9117 bp, synthetic construct
  misc_feature 1..9117: note = nucleic acid construct
  source 1..9117: mol_type = other DNA
gatcatgagcggagaattaagggagtcacgttatgacccccgccgatgacgcgggacaagccgttttacgtttggaactgacagaaccgcaacgttgaaggagccactcagccgcgggtttctggagtttaatgagctaagcacatacgtcagaaaccattattgcgcgttcaaaagtcgcctaaggtcactatcagctagcaaatatttcttgtcaaaaatgctccactgacgttccataaattcccctcggtatccaattagagtctcatattcactctcaatccaaataatctgcaacccagctttcttgtacaaagtggtagctcgaatttccccgatcgttcaaacatttggcaataaagtttcttaagattgaatcctgttgccggtcttgcgatgattatcatataatttctgttgaattacgttaagcatgtaataattaacatgtaatgcatgacgttatttatgagatgggtttttatgattagagtcccgcaattatacatttaatacgcgatagaaaacaaaatatagcgcgcaaactaggataaattatcgcgcgcggtgtcatctatgttactagatcgggaaagcttttaaactatcagtgtttgacaggatatattggcgggtaaacctaagagaaaagagcgtttattagaataatcggatatttaaaagggcgtgaaaaggtttatccgttcgtccatttgtatgtgcatgccaaccacagggttcccctcgggatcaaagtactttgatccaacccctccgctgctatagtgcagtcggcttctgacgttcagtgcagccgtcttctgaaaacgacatgtcgcacaagtcctaagttacgcgacaggctgccgccctgcccttttcctggcgttttcttgtcgcgtgttttagtcgcataaagtagaatacttgcgactagaaccggagacattacgccatgaacaagagcgccgccgctggcctgctgggctatgcccgcgtcagcaccgacgaccaggacttgaccaaccaacgggccgaactgcacgcggccggctgcaccaagctgttttccgagaagatcaccggcaccaggcgcgaccgcccggagctggccaggatgcttgaccacctacgccctggcgacgttgtgacagtgaccaggctagaccgcctggcccgcagcacccgcgacctactggacattgccgagcgcatccaggaggccggcgcgggcctgcgtagcctggcagagccgtgggccgacaccaccacgccggccggccgcatggtgttgaccgtgttcgccggcattgccgagttcgagcgttccctaatcatcgaccgcacccggagcgggcgcgaggccgccaaggcccgaggcgtgaagtttggcccccgccctaccctcaccccggcacagatcgcgcacgcccgcgagctgatcgaccaggaaggccgcaccgtgaaagaggcggctgcactgcttggcgtgcatcgctcgaccctgtaccgcgcacttgagcgcagcgaggaagtgacgcccaccgaggccaggcggcgcggtgccttccgtgaggacgcattgaccgaggccgacgccctggcggccgccgagaatgaacgccaagaggaacaagcatgaaaccgcaccaggacggccaggacgaaccgtttttcattaccgaagagatcgaggcggagatgatcgcggccgggtacgtgttcgagccgcccgcgcacgtctcaaccgtgcggctgcatgaaatcctggccggtttgtctgatgccaagctggcggcctggccggccagcttggccgctgaagaaaccgagcgccgccgtctaaaaaggtgatgtgtatttgagtaaaacagcttgcgtcatgcggtcgctgcgtatatgatgcgatgagtaaataaacaaatacgcaaggggaacgcatgaaggttatcgctgtacttaaccagaaaggcgggtcaggcaagacgaccatcgcaacccatctagcccgcgccctgcaactcgccggggccgatgttctgttagtcgattccgatccccagggcagtgcccgcgattgggcggccgtgcgggaagatcaaccgctaaccgttgtcggcatcgaccgcccgacgattgaccgcgacgtgaaggccatcggccggcgcgacttcgtagtgatcgacggagcgccccaggcggcggacttggctgtgtccgcgatcaaggcagccgacttcgtgctgattccggtgcagccaagcccttacgacatatgggccaccgccgacctggtggagctggttaagcagcgcattgaggtcacggatggaaggctacaagcggcctttgtcgtgtcgcgggcgatcaaaggcacgcgcatcggcggtgaggttgccgaggcgctggccgggtacgagctgcccattcttgagtcccgtatcacgcagcgcgtgagctacccaggcactgccgccgccggcacaaccgttcttgaatcagaacccgagggcgacgctgcccgcgaggtccaggcgctggccgctgaaattaaatcaaaactcatttgagttaatgaggtaaagagaaaatgagcaaaagcacaaacacgctaagtgccggccgtccgagcgcacgcagcagcaaggctgcaacgttggccagcctggcagacacgccagccatgaagcgggtcaactttcagttgccggcggaggatcacaccaagctgaagatgtacgcggtacgccaaggcaagaccattaccgagctgctatctgaatacatcgcgcagctaccagagtaaatgagcaaatgaataaatgagtagatgaattttagcggctaaaggaggcggcatggaaaatcaagaacaaccaggcaccgacgccgtggaatgccccatgtgtggaggaacgggcggttggccaggcgtaagcggctgggttgcctgccggccctgcaatggcactggaacccccaagcccgaggaatcggcgtgagcggtcgcaaaccatccggcccggtacaaatcggcgcggcgctgggtgatgacctggtggagaagttgaaggccgcgcaggccgcccagcggcaacgcatcgaggcagaagcacgccccggtgaatcgtggcaagcggccgctgatcgaatccgcaaagaatcccggcaaccgccggcagccggtgcgccgtcgattaggaagccgcccaagggcgacgagcaaccagattttttcgttccgatgctctatgacgtgggcacccgcgatagtcgcagcatcatggacgtggccgttttccgtctgtcgaagcgtgaccgacgagctggcgaggtgatccgctacgagcttccagacgggcacgtagaggtttccgcagggccggccggcatggccagtgtgtgggattacgacctggtactgatggcggtttcccatctaaccgaatccatgaaccgataccgggaagggaagggagacaagcccggccgcgtgttccgtccacacgttgcggacgtactcaagttctgccggcgagccgatggcggaaagcagaaagacgacctggtagaaacctgcattcggttaaacaccacgcacgttgccatgcagcgtacgaagaaggccaagaacggccgcctggtgacggtatccgagggtgaagccttgattagccgctacaagatcgtaaagagcgaaaccgggcggccggagtacatcgagatcgagctagctgattggatgtaccgcgagatcacagaaggcaagaacccggacgtgctgacggttcaccccgattactttttgatcgatcccggcatcggccgttttctctaccgcctggcacgccgcgccgcaggcaaggcagaagccagatggttgttcaagacgatctacgaacgcagtggcagcgccggagagttcaagaagttctgtttcaccgtgcgcaagctgatcgggtcaaatgacctgccggagtacgatttgaaggaggaggcggggcaggctggcccgatcctagtcatgcgctaccgcaacctgatcgagggcgaagcatccgccggttcctaatgtacggagcagatgctagggcaaattgccctagcaggggaaaaaggtcgaaaaggtctctttcctgtggatagcacgtacattgggaacccaaagccgtacattgggaaccggaacccgtacattgggaacccaaagccgtacattgggaaccggtcacacatgtaagtgactgatataaaagagaaaaaaggcgatttttccgcctaaaactctttaaaacttattaaaactcttaaaacccgcctggcctgtgcataactgtctggccagcgcacagccgaagagctgcaaaaagcgcctacccttcggtcgctgcgctccctacgccccgccgcttcgcgtcggcctatcgcggccgctggccgctcaaaaatggctggcctacggccaggcaatctaccagggcgcggacaagccgcgccgtcgccactcgaccgccggcgcccacatcaaggcaccctgcctcgcgcgtttcggtgatgacggtgaaaacctctgacacatgcagctcccggagacggtcacagcttgtctgtaagcggatgccgggagcagacaagcccgtcagggcgcgtcagcgggtgttggcgggtgtcggggcgcagccatgacccagtcacgtagcgatagcggagtgtatactggcttaactatgcggcatcagagcagattgtactgagagtgcaccatatgcggtgtgaaataccgcacagatgcgtaaggagaaaataccgcatcaggcgctcttccgcttcctcgctcactgactcgctgcgctcggtcgttcggctgcggcgagcggtatcagctcactcaaaggcggtaatacggttatccacagaatcaggggataacgcaggaaagaacatgtgagcaaaaggccagcaaaaggccaggaaccgtaaaaaggccgcgttgctggcgtttttccataggctccgcccccctgacgagcatcacaaaaatcgacgctcaagtcagaggtggcgaaacccgacaggactataaagataccaggcgtttccccctggaagctccctcgtgcgctctcctgttccgaccctgccgcttaccggatacctgtccgcctttctcccttcgggaagcgtggcgctttctcatagctcacgctgtaggtatctcagttcggtgtaggtcgttcgctccaagctgggctgtgtgcacgaaccccccgttcagcccgaccgctgcgccttatccggtaactatcgtcttgagtccaacccggtaagacacgacttatcgccactggcagcagccactggtaacaggattagcagagcgaggtatgtaggcggtgctacagagttcttgaagtggtggcctaactacggctacactagaaggacagtatttggtatctgcgctctgctgaagccagttaccttcggaaaaagagttggtagctcttgatccggcaaacaaaccaccgctggtagcggtggtttttttgtttgcaagcagcagattacgcgcagaaaaaaaggatctcaagaagatcctttgatcttttctacggggtctgacgctcagtggaacgaaaactcacgttaagggattttggtcatgcattctaggtactaaaacaattcatccagtaaaatataatattttattttctcccaatcaggcttgatccccagtaagtcaaaaaatagctcgacatactgttcttccccgatatcctccctgatcgaccggacgcagaaggcaatgtcataccacttgtccgccctgccgcttctcccaagatcaataaagccacttactttgccatctttcacaaagatgttgctgtctcccaggtcgccgtgggaaaagacaagttcctcttcgggcttttccgtctttaaaaaatcatacagctcgcgcggatctttaaatggagtgtcttcttcccagttttcgcaatccacatcggccagatcgttattcagtaagtaatccaattcggctaagcggctgtctaagctattcgtatagggacaatccgatatgtcgatggagtgaaagagcctgatgcactccgcatacagctcgataatcttttcagggctttgttcatcttcatactcttccgagcaaaggacgccatcggcctcactcatgagcagattgctccagccatcatgccgttcaaagtgcaggacctttggaacaggcagctttccttccagccatagcatcatgtccttttcccgttccacatcataggtggtccctttataccggctgtccgtcatttttaaatataggttttcattttctcccaccagcttatataccttagcaggagacattccttccgtatcttttacgcagcggtatttttcgatcagttttttcaattccggtgatattctcattttagccatttattatttccttcctcttttctacagtatttaaagataccccaagaagctaattataacaagacgaactccaattcactgttccttgcattctaaaaccttaaataccagaaaacagctttttcaaagttgttttcaaagttggcgtataacatagtatcgacggagccgattttgaaaccgcggtgatcacaggcagcaacgctctgtcatcgttacaatcaacatgctaccctccgcgagatcatccgtgtttcaaacccggcagcttagttgccgttcttccgaatagcatcggtaacatgagcaaagtctgccgccttacaacggctctcccgctgacgccgtcccggactgatgggctgcctgtatcgagtggtgattttgtgccgagctgccggtcggggagctgttggctggctggtggcaggatatattgtggtgtaaacaaattgacgcttagacaacttaataacacattgcggacgtttttaatgtactgaattaacgccgaattgaattcgagctcggtaccgggggatctggattttagtactggattttggttttaggaattagaaattttattgatagaagtattttacaaatacaaatacatactaagggtttcttatatgctcaacacatgagcgaaaccctataggaaccctaattcccttatctgggaactactcacacattattatggagaaactcgagcttgtcgatcgacagatcccggtcggcatctactctatttctttgccctcggacgagtgctggggcgtcggtttccactatcggcgagtacttctacacagccatcggtccagacggccgcgcttctgcgggcgatttgtgtacgcccgacagtcccggctccggatcggacgattgcgtcgcatcgaccctgcgcccaagctgcatcatcgaaattgccgtcaaccaagctctgatagagttggtcaagaccaatgcggagcatatacgcccggagtcgtggcgatcctgcaagctccggatgcctccgctcgaagtagcgcgtctgctgctccatacaagccaaccacggcctccagaagaagatgttggcgacctcgtattgggaatccccgaacatcgcctcgctccagtcaatgaccgctgttatgcggccattgtccgtcaggacattgttggagccgaaatccgcgtgcacgaggtgccggacttcggggcagtcctcggcccaaagcatcagctcatcgagagcctgcgcgacggacgcactgacggtgtcgtccatcacagtttgccagtgatacacatggggatcagcaatcgcgcatatgaaatcacgccatgtagtgtattgaccgattccttgcggtccgaatgggccgaacccgctcgtctggctaagatcggccgcagcgatcgcatccatagcctccgcgaccggttgtagaacagcgggcagttcggtttcaggcaggtcttgcaacgtgacaccctgtgaacggcgggagatgcaataggtcaggctctcgctaaactccccaatgtcaagcacttccggaatcgggagcgcggccgatgcaaagtgccgataaacataacgatctttgtagaaaccatcggcgcagctatttacccgcaggacatatccacgccctcctacatcgaagctgaaagcacgagattcttcgccctccgagagctgcatcaggtcggagacgctgtcgaacttttcgatcagaaacttctcgacagacgtcgcggtgagttcaggctttttcatatctcattgccccccggatctgcgaaagctcgagagagatagatttgtagagagagactggtgatttcagcgtgtcctctccaaatgaaatgaacttccttatatagaggaagggtcttgcgaaggatagtgggattgtgcgtcatcccttacgtcagtggagatatcacatcaatccacttgctttgaagacgtggttggaacgtcttctttttccacgatgctcctcgtgggtgggggtccatctttgggaccactgtcggcagaggcatcttgaacgatagcctttcctttatcgcaatgatggcatttgtaggtgccaccttccttttctactgtccttttgatgaagtgacagatagctgggcaatggaatccgaggaggtttcccgatattaccctttgttgaaaagtctcaatagccctttggtcttctgagactgtatctttgatattcttggagtagacgagagtgtcgtgctccaccatgttcacatcaatccacttgctttgaagacgtggttggaacgtcttctttttccacgatgctcctcgtgggtgggggtccatctttgggaccactgtcggcagaggcatcttgaacgatagcctttcctttatcgcaatgatggcatttgtaggtgccaccttccttttctactgtccttttgatgaagtgacagatagctgggcaatggaatccgaggaggtttcccgatattaccctttgttgaaaagtctcaatagccctttggtcttctgagactgtatctttgatattcttggagtagacgagagtgtcgtgctccaccatgttggcgtacccggggatcctctagagtcgacctgcaggcatgcaagct